European Patent Application EP 4 501 951 A2, published February 5, 2025. Title: T CELLS WITH IMPROVED FUNCTIONALITY. Applicant: Kite Pharma, Inc. Application EP. The sequence listing filed with the application follows.

SEQUENCE LISTING (14 sequences)

SEQ ID NO: 1 - protein, 6 aa, Porcine teschovirus
CHYSEL

SEQ ID NO: 2 - protein, 8 aa, synthetic construct
DXEXNPGP

SEQ ID NO: 3 - protein, 9 aa, synthetic construct
LAGLIDADG

SEQ ID NO: 4 - protein, 389 aa, Homo sapiens
MPQLDSGGGGAGGGDDLGAPDELLAFQDEGEEQDDKSRDSAAGPERDLAELKSSLVNESEGAAGGAGIPGVPGAGAGARGEAEALGREHAAQRLFPDKLPEPLEDGLKAPECTSGMYKETVYSAFNLLMHYPPPSGAGQHPQPQPPLHKANQPPHGVPQLSLYEHFNSPHPTPAPADISQKQVHRPLQTPDLSGFYSLTSGSMGQLPHTVSWFTHPSLMLGSGVPGHPAAIPHPAIVPPSGKQELQPFDRNLKTQAESKAEKEAKKPTIKKPLNAFMLYMKEMRAKVIAECTLKESAAINQILGRRWHALSREEQAKYYELARKERQLHMQLYPGWSARDNYGKKKRRSREKHQESTTGGKRNAFGTYPEKAAAPAPFLPMTVLRAKRS

SEQ ID NO: 5 - DNA, 1167 bp, Homo sapiens
  source 1..1167: mol_type = other DNA
atgcctcagctggattctggcggaggcggagctggtggcggagatgatcttggagcacctgatgagctgctggcattccaggacgagggcgaagaacaggacgacaagagcagagattctgccgccggacctgagagagatctggccgagctgaagtccagcctggtcaatgaatctgaaggcgccgctggcggcgctggaattcctggtgttcctggcgctggtgctggtgcaagaggcgaagctgaagccctgggaagagaacacgctgcccagagactgttccccgacaagctgcctgagcctctggaagatggactgaaggcccctgagtgtaccagcggcatgtacaaagaaaccgtgtacagcgccttcaacctgctgatgcactaccctccacctagcggagcaggacagcatcctcaacctcagcctccactgcacaaggccaatcagccacctcatggcgtgccacagctgagcctgtacgagcacttcaacagccctcatcctactccagctccagccgacatcagccagaaacaggtgcacagacctctgcagacccctgacctgagcggcttttacagcctgacaagcggcagcatgggacagctgcctcataccgtgtcctggttcacacaccccagcctgatgcttggaagcggagtgcctggacaccctgccgctattcctcatcctgccatcgtgcctccaagcggcaagcaagagctgcagcccttcgaccggaacctgaaaacacaggccgagagcaaggccgagaaagaggccaagaagcccaccatcaagaagcctctgaacgccttcatgctgtacatgaaagaaatgcgggccaaagtgatcgccgagtgcaccctgaaagagtccgccgccatcaaccagatcctgggcagaagatggcacgccctgtccagagaggaacaggccaagtactacgagctggcccggaaagaacggcagctgcacatgcaactgtaccctggctggagcgccagagacaactacggcaagaagaagcggcggagcagagagaagcaccaagagtctacaaccggcggcaagagaaacgccttcggcacatatcccgagaaagccgctgctcccgctcctttcctgcctatgactgtgctgagggccaagagaagc

SEQ ID NO: 6 - protein, 684 aa, Homo sapiens
MPQLDSGGGGAGGGDDLGAPDELLAFQDEGEEQDDKSRDSAAGPERDLAELKSSLVNESEGAAGGAGIPGVPGAGAGARGEAEALGREHAAQRLFPDKLPEPLEDGLKAPECTSGMYKETVYSAFNLLMHYPPPSGAGQHPQPQPPLHKANQPPHGVPQLSLYEHFNSPHPTPAPADISQKQVHRPLQTPDLSGFYSLTSGSMGQLPHTVSWFTHPSLMLGSGVPGHPAAIPHPAIVPPSGKQELQPFDRNLKTQAESKAEKEAKKPTIKKPLNAFMLYMKEMRAKVIAECTLKESAAINQILGRRWHALSREEQAKYYELARKERQLHMQLYPGWSARDNYGKKKRRSREKHQESTTGGKRNAFGTYPEKAAAPAPFLPMTVLRAKRSGSGEGRGSLLTCGDVEENPGPMGAGATGRAMDGPRLLLLLLLGVSLGGAKEACPTGLYTHSGECCKACNLGEGVAQPCGANQTVCEPCLDSVTFSDVVSATEPCKPCTECVGLQSMSAPCVEADDAVCRCAYGYYQDETTGRCEACRVCEAGSGLVFSCQDKQNTVCEECPDGTYSDEANHVDPCLPCTVCEDTERQLRECTRWADAECEEIPGRWITRSTPPEGSDSTAPSTQEPEAPPEQDLIASTVAGVVTTVMGSSQPVVTRGTTDNLIPVYCSILAAVVVGLVAYIAFKR

SEQ ID NO: 7 - DNA, 2061 bp, Homo sapiens
  source 1..2061: mol_type = other DNA
atgcctcagctggattctggcggaggcggagctggtggcggagatgatcttggagcacctgatgagctgctggcattccaggacgagggcgaagaacaggacgacaagagcagagattctgccgccggacctgagagagatctggccgagctgaagtccagcctggtcaatgaatctgaaggcgccgctggcggcgctggaattcctggtgttcctggcgctggtgctggtgcaagaggcgaagctgaagccctgggaagagaacacgctgcccagagactgttccccgacaagctgcctgagcctctggaagatggactgaaggcccctgagtgtaccagcggcatgtacaaagaaaccgtgtacagcgccttcaacctgctgatgcactaccctccacctagcggagcaggacagcatcctcaacctcagcctccactgcacaaggccaatcagccacctcatggcgtgccacagctgagcctgtacgagcacttcaacagccctcatcctactccagctccagccgacatcagccagaaacaggtgcacagacctctgcagacccctgacctgagcggcttttacagcctgacaagcggcagcatgggacagctgcctcataccgtgtcctggttcacacaccccagcctgatgcttggaagcggagtgcctggacaccctgccgctattcctcatcctgccatcgtgcctccaagcggcaagcaagagctgcagcccttcgaccggaacctgaaaacacaggccgagagcaaggccgagaaagaggccaagaagcccaccatcaagaagcctctgaacgccttcatgctgtacatgaaagaaatgcgggccaaagtgatcgccgagtgcaccctgaaagagtccgccgccatcaaccagatcctgggcagaagatggcacgccctgtccagagaggaacaggccaagtactacgagctggcccggaaagaacggcagctgcacatgcaactgtaccctggctggagcgccagagacaactacggcaagaagaagcggcggagcagagagaagcaccaagagtctacaaccggcggcaagagaaacgccttcggcacatatcccgagaaagccgctgctcccgctcctttcctgcctatgactgtgctgagggccaagagaagcggaagtggagagggaagaggctcccttctgacatgcggcgacgtggaggagaaccctggacctatgggagctggagctaccggaagagctatggacggaccaagacttctcctgctcctcctgctgggtgtgagcctgggaggagctaaggaggcttgccctaccggactgtacacccactctggcgagtgctgcaaggcttgcaacctgggagagggagtggctcaaccctgcggagctaaccaaactgtctgcgagccttgcctggactctgtgacattctccgacgtggtgtctgccaccgagccttgcaagccttgcaccgaatgcgtgggcctgcaaagcatgagcgctccttgcgtggaggctgacgacgctgtgtgccgatgcgcttacggatactaccaagacgagaccaccggaagatgcgaggcttgccgagtgtgcgaggctggaagcggactcgtgttctcctgccaagacaagcaaaacaccgtgtgtgaggaatgccctgacggaacctactccgacgaggctaaccacgtggacccttgcctgccttgcaccgtgtgtgaggacaccgagagacaactgagggagtgcacaagatgggctgacgctgagtgtgaggagatccctggaagatggatcacaagatctacccctcctgagggaagcgactccaccgctccttccacccaagagcccgaggctcctcctgagcaagacctgatcgcaagcaccgtggctggagtggttacaaccgtgatgggaagctcccaacccgtggttacaaggggaaccaccgacaacctgatccctgtgtactgctccatcctggctgctgtggtggtgggattggtggcctacatcgctttcaagagatgaatcgat

SEQ ID NO: 8 - protein, 846 aa, Homo sapiens
MSVDEKPDSPMYVYESTVHCTNILLGLNDQRKKDILCDVTLIVERKEFRAHRAVLAACSEYFWQALVGQTKNDLVVSLPEEVTARGFGPLLQFAYTAKLLLSRENIREVIRCAEFLRMHNLEDSCFSFLQTQLLNSEDGLFVCRKDAACQRPHEDCENSAGEEEDEEEETMDSETAKMACPRDQMLPEPISFEAAAIPVAEKEEALLPEPDVPTDTKESSEKDALTQYPRYKKYQLACTKNVYNASSHSTSGFASTFREDNSSNSLKPGLARGQIKSEPPSEENEEESITLCLSGDEPDAKDRAGDVEMDRKQPSPAPTPTAPAGAACLERSRSVASPSCLRSLFSITKSVELSGLPSTSQQHFARSPACPFDKGITQGDLKTDYTPFTGNYGQPHVGQKEVSNFTMGSPLRGPGLEALCKQEGELDRRSVIFSSSACDQVSTSVHSYSGVSSLDKDLSEPVPKGLWVGAGQSLPSSQAYSHGGLMADHLPGRMRPNTSCPVPIKVCPRSPPLETRTRTSSSCSSYSYAEDGSGGSPCSLPLCEFSSSPCSQGARFLATEHQEPGLMGDGMYNQVRPQIKCEQSYGTNSSDESGSFSEADSESCPVQDRGQEVKLPFPVDQITDLPRNDFQMMIKMHKLTSEQLEFIHDVRRRSKNRIAAQRCRKRKLDCIQNLECEIRKLVCEKEKLLSERNQLKACMGELLDNFSCLSQEVCRDIQSPEQIQALHRYCPVLRPMDLPTASSINPAPLGAEQNIAASQCAVGENVPCCLEPGAAPPGPPWAPSNTSENCTSGRRLEGTDPGTFSERGPPLEPRSQTVTVDFCQEMTDKCTTDEQPRKDYTRAKRS

SEQ ID NO: 9 - DNA, 2538 bp, Homo sapiens
  source 1..2538: mol_type = other DNA
atgagcgtggacgagaagcctgacagccctatgtacgtgtacgagagcaccgtgcactgcaccaacatcctgctgggcctgaacgaccagcggaagaaagacatcctgtgcgacgtgaccctgatcgtggaacggaaagagttcagagcccacagagccgtgctggccgcctgtagcgagtatttttggcaggccctcgtgggccagaccaagaacgatctggtggtgtccctgcctgaggaagtgaccgccagaggatttggacccctgctgcagtttgcctacaccgccaaactgctgctgagccgcgagaacatccgggaagtgatcagatgcgccgagttcctgcggatgcacaacctggaagatagctgcttcagcttcctgcagacccagctgctgaacagcgaggatggcctgttcgtgtgcagaaaggatgccgcctgtcagaggcctcacgaggactgcgaaaattctgccggcgaggaagaggacgaagaggaagaaaccatggacagcgagacagccaagatggcttgccccagggaccagatgctgcctgagcctatctctttcgaggccgctgccattcctgtggccgagaaagaagaagccctgctgccagagccagacgtgcccaccgatacaaaagagagcagcgagaaggacgccctgacacagtaccccagatacaagaagtaccagctggcctgcaccaagaatgtgtacaacgccagcagccacagcaccagcggctttgcctctaccttcagagaggacaacagcagcaacagcctgaagcctggactggccagaggccagatcaagtctgagcctcctagcgaggaaaatgaagaggaatctatcaccctgtgcctgagcggcgacgagcctgatgccaaagatagagctggcgacgtggaaatggaccggaagcagccttctccagctcctacacctacagctccagctggcgcagcctgcctggaaagatcaagatctgtggctagccccagctgcctgcggagcctgtttagcatcaccaagagcgtggaactgagcggcctgcctagcacatcccagcagcactttgccagatctcccgcctgtcctttcgacaagggaatcacccagggcgacctgaaaaccgactacacccctttcaccggcaactacggacagcctcacgtgggacagaaagaggtgtccaactttaccatgggcagccctctgagaggcccaggacttgaggccctgtgtaaacaagagggcgagctggatcggcggagcgtgatcttttctagcagcgcctgtgaccaggtgtccaccagcgtgcactcttacagcggagtgtccagcctggataaggacctgtctgagcccgtgcctaaaggcctgtgggttggagctggacagagcctgccaagcagccaggcttattctcacggcggactgatggccgatcatctgcctggtagaatgcggcccaacaccagctgtcccgtgccaatcaaagtgtgccctagaagccctcctctggaaacccggaccagaaccagcagcagctgttccagctacagctatgccgaggatggaagcggcggcagcccttgttcactgcctctgtgcgagtttagcagcagcccctgttctcagggcgccagatttctggccaccgagcatcaagaacctggcctgatgggcgacggcatgtacaatcaagtgcggccccagattaagtgcgagcagagctacggcaccaacagctctgatgagagcggcagctttagcgaggccgatagcgaaagctgccccgtgcaggatagaggccaagaagtgaagctgccctttccagtggatcagatcaccgacctgcctcggaacgacttccagatgatgatcaagatgcacaagctgacctccgagcagctggaattcatccacgacgtgcggcggagaagcaagaacagaatcgctgcccagcggtgccggaagagaaagctggactgcatccagaatctggaatgcgagatccggaagctcgtgtgcgaaaaagagaagctgctgtccgagcggaaccagctgaaggcctgtatgggagagctgctggacaacttcagctgtctgtctcaagaagtgtgccgggacatccagtctccagagcagattcaggccctgcacagatactgccctgtgctgaggcctatggatctgcctacagccagcagcatcaaccctgctcctctgggagccgagcagaatattgccgcctctcagtgtgccgtgggcgagaatgtgccttgctgtcttgaacctggcgccgctcctcctggacctccttgggctccttctaacaccagcgagaactgcacctccggcagaaggctggaaggcacagatcctggcaccttcagcgaaagaggcccaccactggaacccagatctcagaccgtgaccgtggacttctgccaagagatgaccgacaagtgcaccaccgacgagcagcccagaaaggactacaccagggccaagagaagc

SEQ ID NO: 10 - protein, 1141 aa, Homo sapiens
MSVDEKPDSPMYVYESTVHCTNILLGLNDQRKKDILCDVTLIVERKEFRAHRAVLAACSEYFWQALVGQTKNDLVVSLPEEVTARGFGPLLQFAYTAKLLLSRENIREVIRCAEFLRMHNLEDSCFSFLQTQLLNSEDGLFVCRKDAACQRPHEDCENSAGEEEDEEEETMDSETAKMACPRDQMLPEPISFEAAAIPVAEKEEALLPEPDVPTDTKESSEKDALTQYPRYKKYQLACTKNVYNASSHSTSGFASTFREDNSSNSLKPGLARGQIKSEPPSEENEEESITLCLSGDEPDAKDRAGDVEMDRKQPSPAPTPTAPAGAACLERSRSVASPSCLRSLFSITKSVELSGLPSTSQQHFARSPACPFDKGITQGDLKTDYTPFTGNYGQPHVGQKEVSNFTMGSPLRGPGLEALCKQEGELDRRSVIFSSSACDQVSTSVHSYSGVSSLDKDLSEPVPKGLWVGAGQSLPSSQAYSHGGLMADHLPGRMRPNTSCPVPIKVCPRSPPLETRTRTSSSCSSYSYAEDGSGGSPCSLPLCEFSSSPCSQGARFLATEHQEPGLMGDGMYNQVRPQIKCEQSYGTNSSDESGSFSEADSESCPVQDRGQEVKLPFPVDQITDLPRNDFQMMIKMHKLTSEQLEFIHDVRRRSKNRIAAQRCRKRKLDCIQNLECEIRKLVCEKEKLLSERNQLKACMGELLDNFSCLSQEVCRDIQSPEQIQALHRYCPVLRPMDLPTASSINPAPLGAEQNIAASQCAVGENVPCCLEPGAAPPGPPWAPSNTSENCTSGRRLEGTDPGTFSERGPPLEPRSQTVTVDFCQEMTDKCTTDEQPRKDYTRAKRSGSGEGRGSLLTCGDVEENPGPMGAGATGRAMDGPRLLLLLLLGVSLGGAKEACPTGLYTHSGECCKACNLGEGVAQPCGANQTVCEPCLDSVTFSDVVSATEPCKPCTECVGLQSMSAPCVEADDAVCRCAYGYYQDETTGRCEACRVCEAGSGLVFSCQDKQNTVCEECPDGTYSDEANHVDPCLPCTVCEDTERQLRECTRWADAECEEIPGRWITRSTPPEGSDSTAPSTQEPEAPPEQDLIASTVAGVVTTVMGSSQPVVTRGTTDNLIPVYCSILAAVVVGLVAYIAFKR

SEQ ID NO: 11 - DNA, 3432 bp, Homo sapiens
  source 1..3432: mol_type = other DNA
atgagcgtggacgagaagcctgacagccctatgtacgtgtacgagagcaccgtgcactgcaccaacatcctgctgggcctgaacgaccagcggaagaaagacatcctgtgcgacgtgaccctgatcgtggaacggaaagagttcagagcccacagagccgtgctggccgcctgtagcgagtatttttggcaggccctcgtgggccagaccaagaacgatctggtggtgtccctgcctgaggaagtgaccgccagaggatttggacccctgctgcagtttgcctacaccgccaaactgctgctgagccgcgagaacatccgggaagtgatcagatgcgccgagttcctgcggatgcacaacctggaagatagctgcttcagcttcctgcagacccagctgctgaacagcgaggatggcctgttcgtgtgcagaaaggatgccgcctgtcagaggcctcacgaggactgcgaaaattctgccggcgaggaagaggacgaagaggaagaaaccatggacagcgagacagccaagatggcttgccccagggaccagatgctgcctgagcctatctctttcgaggccgctgccattcctgtggccgagaaagaagaagccctgctgccagagccagacgtgcccaccgatacaaaagagagcagcgagaaggacgccctgacacagtaccccagatacaagaagtaccagctggcctgcaccaagaatgtgtacaacgccagcagccacagcaccagcggctttgcctctaccttcagagaggacaacagcagcaacagcctgaagcctggactggccagaggccagatcaagtctgagcctcctagcgaggaaaatgaagaggaatctatcaccctgtgcctgagcggcgacgagcctgatgccaaagatagagctggcgacgtggaaatggaccggaagcagccttctccagctcctacacctacagctccagctggcgcagcctgcctggaaagatcaagatctgtggctagccccagctgcctgcggagcctgtttagcatcaccaagagcgtggaactgagcggcctgcctagcacatcccagcagcactttgccagatctcccgcctgtcctttcgacaagggaatcacccagggcgacctgaaaaccgactacacccctttcaccggcaactacggacagcctcacgtgggacagaaagaggtgtccaactttaccatgggcagccctctgagaggcccaggacttgaggccctgtgtaaacaagagggcgagctggatcggcggagcgtgatcttttctagcagcgcctgtgaccaggtgtccaccagcgtgcactcttacagcggagtgtccagcctggataaggacctgtctgagcccgtgcctaaaggcctgtgggttggagctggacagagcctgccaagcagccaggcttattctcacggcggactgatggccgatcatctgcctggtagaatgcggcccaacaccagctgtcccgtgccaatcaaagtgtgccctagaagccctcctctggaaacccggaccagaaccagcagcagctgttccagctacagctatgccgaggatggaagcggcggcagcccttgttcactgcctctgtgcgagtttagcagcagcccctgttctcagggcgccagatttctggccaccgagcatcaagaacctggcctgatgggcgacggcatgtacaatcaagtgcggccccagattaagtgcgagcagagctacggcaccaacagctctgatgagagcggcagctttagcgaggccgatagcgaaagctgccccgtgcaggatagaggccaagaagtgaagctgccctttccagtggatcagatcaccgacctgcctcggaacgacttccagatgatgatcaagatgcacaagctgacctccgagcagctggaattcatccacgacgtgcggcggagaagcaagaacagaatcgctgcccagcggtgccggaagagaaagctggactgcatccagaatctggaatgcgagatccggaagctcgtgtgcgaaaaagagaagctgctgtccgagcggaaccagctgaaggcctgtatgggagagctgctggacaacttcagctgtctgtctcaagaagtgtgccgggacatccagtctccagagcagattcaggccctgcacagatactgccctgtgctgaggcctatggatctgcctacagccagcagcatcaaccctgctcctctgggagccgagcagaatattgccgcctctcagtgtgccgtgggcgagaatgtgccttgctgtcttgaacctggcgccgctcctcctggacctccttgggctccttctaacaccagcgagaactgcacctccggcagaaggctggaaggcacagatcctggcaccttcagcgaaagaggcccaccactggaacccagatctcagaccgtgaccgtggacttctgccaagagatgaccgacaagtgcaccaccgacgagcagcccagaaaggactacaccagggccaagagaagcggaagtggagagggaagaggctcccttctgacatgcggcgacgtggaggagaaccctggacctatgggagctggagctaccggaagagctatggacggaccaagacttctcctgctcctcctgctgggtgtgagcctgggaggagctaaggaggcttgccctaccggactgtacacccactctggcgagtgctgcaaggcttgcaacctgggagagggagtggctcaaccctgcggagctaaccaaactgtctgcgagccttgcctggactctgtgacattctccgacgtggtgtctgccaccgagccttgcaagccttgcaccgaatgcgtgggcctgcaaagcatgagcgctccttgcgtggaggctgacgacgctgtgtgccgatgcgcttacggatactaccaagacgagaccaccggaagatgcgaggcttgccgagtgtgcgaggctggaagcggactcgtgttctcctgccaagacaagcaaaacaccgtgtgtgaggaatgccctgacggaacctactccgacgaggctaaccacgtggacccttgcctgccttgcaccgtgtgtgaggacaccgagagacaactgagggagtgcacaagatgggctgacgctgagtgtgaggagatccctggaagatggatcacaagatctacccctcctgagggaagcgactccaccgctccttccacccaagagcccgaggctcctcctgagcaagacctgatcgcaagcaccgtggctggagtggttacaaccgtgatgggaagctcccaacccgtggttacaaggggaaccaccgacaacctgatccctgtgtactgctccatcctggctgctgtggtggtgggattggtggcctacatcgctttcaagagatgaatcgat

SEQ ID NO: 12 - RNA, 20 nt, synthetic construct
  source 1..20: mol_type = other RNA
gaagtggtgaagctcccctc

SEQ ID NO: 13 - RNA, 20 nt, synthetic construct
  source 1..20: mol_type = other RNA
ctctccccgggagcaaaacc

SEQ ID NO: 14 - RNA, 20 nt, synthetic construct
  source 1..20: mol_type = other RNA
gttggcagggatgggcttaa